European Patent Application EP 4 582 447 A1, published July 9, 2025. Title: ANTI-VEGFA ANTIBODY OR ANTIGEN-BINDING FRAGMENT THEREOF AND USE THEREOF. Applicant: Quaerite Biopharm Research (Beijing) Co., Ltd. The sequence listing filed with the application follows.

SEQUENCE LISTING (75 sequences)

SEQ ID NO: 1 - protein, 5 aa, synthetic construct
SYTMG

SEQ ID NO: 2 - protein, 16 aa, synthetic construct
  SITE 10..11: note = XX can be DS, DA, NT, DT, NA or NS
AISKGGYKYXXVSLEA

SEQ ID NO: 3 - protein, 17 aa, synthetic construct
  SITE 10: note = R or K
  SITE 13: note = D, N, E or K
TRAYGSSRLXLAXTYEY

SEQ ID NO: 4 - protein, 16 aa, synthetic construct
AISKGGYKYDSVSLEA

SEQ ID NO: 5 - protein, 16 aa, synthetic construct
AISKGGYKYDAVSLEA

SEQ ID NO: 6 - protein, 16 aa, synthetic construct
AISKGGYKYNTVSLEA

SEQ ID NO: 7 - protein, 16 aa, synthetic construct
AISKGGYKYDTVSLEA

SEQ ID NO: 8 - protein, 16 aa, synthetic construct
AISKGGYKYNAVSLEA

SEQ ID NO: 9 - protein, 17 aa, synthetic construct
TRAYGSSRLRLADTYEY

SEQ ID NO: 10 - protein, 17 aa, synthetic construct
TRAYGSSRLRLANTYEY

SEQ ID NO: 11 - protein, 17 aa, synthetic construct
TRAYGSSRLRLAETYEY

SEQ ID NO: 12 - protein, 17 aa, synthetic construct
TRAYGSSRLRLAKTYEY

SEQ ID NO: 13 - protein, 125 aa, synthetic construct
QLQLVESGGGSVQPGGSLRLSCEVSGRTFSSYTMGWFRQAPGKEREFVVAISKGGYKYDSVSLEARFTISKDNTKNTVYLQMNSLKPEDTAVYYCAATRAYGSSRLRLADTYEYWGQGTQVTVSS

SEQ ID NO: 14 - protein, 125 aa, synthetic construct
QLQLVESGGGSVQPGGSLRLSCEVSGRTFSSYTMGWFRQAPGKEREFVVAISKGGYKYDTVSLEARFTISKDNTKNTVYLQMNSLKPEDTAVYYCAGTRAYGSSRLKLADTYEYWGQGTQVTVSS

SEQ ID NO: 15 - protein, 125 aa, synthetic construct
QLQLVESGGGSVQPGGSLRLSCEVSGRTFSSYTMGWFRQAPGKEREFVVAISKGGYKYNTVSLEARFTISKDNTKNTVYLQMNSLKPEDTAVYYCAGTRAYGSSRLKLAETYEYWGQGTQVTVSS

SEQ ID NO: 16 - protein, 125 aa, synthetic construct
QLQLVESGGGSVQPGGSLRLSCEVSGRTFTSYTMGWFRQAPGKEREFVVAISKGGYKYDAVSLEARFTISKDNTKNTVYLQMNSLKPEDTAVYYCAGTRAYGSSRLRLADTYEYWGQGTQVTVSS

SEQ ID NO: 17 - protein, 125 aa, synthetic construct
QLQLVESGGGSVQPGGSLRLSCEVSGRTFTSYTMGWFRQAPGKEREFVVAISKGGYKYNTVSLEARFTISKDNTKNTVYLQMNSLKPEDTAVYYCAGTRAYGSSRLRLANTYEYWGQGTQVTVSS

SEQ ID NO: 18 - protein, 125 aa, synthetic construct
QLQLVESGGGSVQPGGSLRLSCEVSGRTFASYTMGWFRQAPGKEREFVVAISKGGYKYDSVSLEARFTISKDNTKNTVYLQMNSLKPEDTAVYYCAGTRAYGSSRLRLAETYEYWGQGTQVTVSS

SEQ ID NO: 19 - protein, 125 aa, synthetic construct
QLQLVESGGGSVQPGGSLRLSCEVSGRTFSSYTMGWFRQAPGKEREFVVAISKGGYKYDTVSLEARFTISKDNTKNTVYLQMNSLKPEDTAVYYCAATRAYGSSRLRLAKTYEYWGQGTQVTVSS

SEQ ID NO: 20 - protein, 125 aa, synthetic construct
QLQLVESGGGSVQPGGSLRLSCEVSGRTFSSYTMGWFRQAPGKEREFVVAISKGGYKYNSVSLEARFTISKDNTKNTVYLQMNSLKPEDTAVYYCAGTRAYGSSRLRLADTYEYWGQGTQVTVSS

SEQ ID NO: 21 - protein, 125 aa, synthetic construct
QLQLVESGGGSVQPGGSLRLSCEVSGRTFSSYTMGWFRQAPGKEREFVVAISKGGYKYNSVSLEARFTISKDNTKNTVYLQMNSLKPEDTAVYYCAATRAYGSSRLKLANTYEYWGQGTQVTVSS

SEQ ID NO: 22 - protein, 125 aa, synthetic construct
QLQLVESGGGSVQPGGSLRLSCEVSGRTFTSYTMGWFRQAPGKEREFVVAISKGGYKYNTVSLEARFTISKDNTKNTVYLQMNSLKPEDTAVYYCAGTRAYGSSRLRLAETYEYWGQGTQVTVSS

SEQ ID NO: 23 - protein, 125 aa, synthetic construct
QLQLVESGGGSVQPGGSLRLSCEVSGRTFSSYTMGWFRQAPGKEREFVVAISKGGYKYDSVSLEARFTISKDNTKNTVYLQMNSLKPEDTAVYYCAATRAYGSSRLKLADTYEYWGQGTQVTVSS

SEQ ID NO: 24 - protein, 125 aa, synthetic construct
QLQLVESGGGSVQPGGSLRLSCEVSGRTFTSYTMGWFRRAPGKEREFVVAISKGGYKYDSVSLEARFTISKDNTKNTVYLQMNSLKPEDTAVYYCAGTRAYGSSRLKLAKTYEYWGQGTQVTVSS

SEQ ID NO: 25 - protein, 125 aa, synthetic construct
QLQLVESGGGSVQPGGSLRLSCEVSGRTFSSYTMGWFRQAPGKEREFVVAISKGGYKYDSVSLEARFTISKDNTKNTVYLQMNSLKPEDTAVYYCAGTRAYGSSRLRLANTYEYWGQGTQVTVSS

SEQ ID NO: 26 - protein, 125 aa, synthetic construct
QLQLVESGGGSVQPGGSLRLSCEVSGRTFSSYTMGWFRQAPGKGREFVVAISKGGYKYDAVSLEARFTISKDNTKNTVYLQMNSLKPEDTAVYYCAATRAYGSSRLRLAKTYEYWGQGTQVTVSS

SEQ ID NO: 27 - protein, 125 aa, synthetic construct
QLQLVESGGGSVQPGGSLRLSCEVSGRTFASYTMGWFRQAPGKEREFVVAISKGGYKYDAVSLEARFTISKDNTKNTVYLQMNSLKPEDTAVYYCAGTRAYGSSRLRLAKTYEYWGQGTQVTVSS

SEQ ID NO: 28 - protein, 125 aa, synthetic construct
QLQLVESGGGSVQPGGSLRLSCEVSGRTFSSYTMGWFRQAPGKEREFVVAISKGGYKYDSVSLEARFTISKDNTKNTVYLQMNSLKPEDTAVYYCAATRAYGSSRLRLAKTYEYWGQGTQVTVSS

SEQ ID NO: 29 - protein, 125 aa, synthetic construct
QLQLVESGGGSVQPGGSLRLSCEVSGRTFASYTMGWFRQAPGKEREFVVAISKGGYKYDSVSLEARFTISKDNTKNTVYLQMNSLKPEDTAVYYCAGTRAYGSSRLRLADTYEYWGQGTQVTVSS

SEQ ID NO: 30 - protein, 125 aa, synthetic construct
QLQLVESGGGSVQPGGSLRLSCEVSGRTFTSYTMGWFRQAPGKEREFVVAISKGGYKYNAVSLEARFTISKDNTKNTVYLQMNSLKPEDTAVYYCAGTRAYGSSRLRLAKTYEYWGQGTQVTVSS

SEQ ID NO: 31 - protein, 125 aa, synthetic construct
QLQLVESGGGSVQPGGSLRLSCEVSGRTFSSYTMGWFRQAPGKEREFVVAISKGGYKYDSVSLEARFTISKDNTKNTVYLQMNSLKPEDTAVYYCAGTRAYGSSRLRLAKTYEYWGQGTQVTVSS

SEQ ID NO: 32 - protein, 125 aa, synthetic construct
QLQLVESGGGSVQPGGSLRLSCEVSGRTFTSYTMGWFRQAPGKEREFVVAISKGGYKYDSVSLEARFTISKDNTKNTVYLQMNSLKPEDTAVYYCAGTRAYGSSRLRLANTYEYWGQGTQVTVSS

SEQ ID NO: 33 - protein, 16 aa, synthetic construct
AISKGGYKYNSVSLEA

SEQ ID NO: 34 - protein, 17 aa, synthetic construct
TRAYGSSRLKLANTYEY

SEQ ID NO: 35 - protein, 125 aa, synthetic construct
EVQLVESGGGLVQPGGSLRLSCAASGRTFSSYTMGWFRQAPGKEREFVVAISKGGYKYDSVSLEARFTISRDNSKNTVYLQMNSLRAEDTAVYYCAATRAYGSSRLRLADTYEYWGQGTLVTVSS

SEQ ID NO: 36 - protein, 125 aa, synthetic construct
EVQLVESGGGLVQPGGSLRLSCAASGRTFSSYTMGWFRQAPGKEREFVVAISKGGYKYDSVSLEARFTISRDNSKNTLYLQMNSLRPEDTAVYYCAATRAYGSSRLRLADTYEYWGQGTLVTVSS

SEQ ID NO: 37 - protein, 125 aa, synthetic construct
EVQLVESGGGLVQPGGSLRLSCAASGRTFSSYTMGWFRQAPGKEREFVVAISKGGYKYDSVSLEARFTISRDNSKNTVYLQMNSLRPEDTAVYYCAATRAYGSSRLRLADTYEYWGQGTLVTVSS

SEQ ID NO: 38 - protein, 125 aa, synthetic construct
EVQLVESGGGLVQPGGSLRLSCAASGRTFSSYTMGWFRQAPGKEREFVVAISKGGYKYDSVSLEARFTISRDNAKNTVYLQMNSLRPEDTAVYYCAATRAYGSSRLRLADTYEYWGQGTLVTVSS

SEQ ID NO: 39 - protein, 125 aa, synthetic construct
EVQLVESGGGLVQPGGSLRLSCAASGRTFSSYTMGWFRQAPGKEREFVVAISKGGYKYDSVSLEARFTISRDNAKNTVYLQMNSLRAEDTAVYYCASTRAYGSSRLRLADTYEYWGQGTLVTVSS

SEQ ID NO: 40 - protein, 125 aa, synthetic construct
EVQLVESGGGLVQPGGSLRLSCAASGRTFSSYTMGWFRQAPGKEREFVVAISKGGYKYDSVSLEARFTISRDNAKNTVYLQMNSLRPEDTAVYYCASTRAYGSSRLRLADTYEYWGQGTLVTVSS

SEQ ID NO: 41 - protein, 125 aa, synthetic construct
EVQLVESGGGLVQPGGSLRLSCAVSGRTFSSYTMGWFRQAPGKEREFVVAISKGGYKYDSVSLEARFTISRDNAKNTVYLQMNSLRPEDTAVYYCAATRAYGSSRLRLADTYEYWGQGTLVTVSS

SEQ ID NO: 42 - protein, 125 aa, synthetic construct
EVQLVESGGGLVQPGGSLRLSCAASGRTFSSYTMGWFRQAPGKEREFVVAISKGGYKYDSVSLEARFTISRDNAKNTVYLQMNSLRAEDTAVYYCAATRAYGSSRLRLADTYEYWGQGTLVTVSS

SEQ ID NO: 43 - protein, 125 aa, synthetic construct
EVQLVESGGGLVQPGGSLRLSCAVSGRTFSSYTMGWFRQAPGKEREFVVAISKGGYKYDSVSLEARFTISRDNSKNTVYLQMNSLRPEDTAVYYCAATRAYGSSRLRLADTYEYWGQGTLVTVSS

SEQ ID NO: 44 - protein, 125 aa, synthetic construct
EVQLVESGGGLVQPGGSLRLSCAASGRTFTSYTMGWFRQAPGKEREFVVAISKGGYKYDAVSLEARFTISRDNSKNTVYLQMNSLRPEDTAVYYCAGTRAYGSSRLRLADTYEYWGQGTLVTVSS

SEQ ID NO: 45 - protein, 125 aa, synthetic construct
EVQLVESGGGLVQPGGSLRLSCAASGRTFTSYTMGWFRQAPGKEREFVVAISKGGYKYDAVSLEARFTISRDNAKNTVYLQMNSLRPEDTAVYYCAGTRAYGSSRLRLADTYEYWGQGTLVTVSS

SEQ ID NO: 46 - protein, 125 aa, synthetic construct
EVQLVESGGGLVQPGGSLRLSCAASGRTFASYTMGWFRQAPGKEREFVVAISKGGYKYDSVSLEARFTISRDNSKNTVYLQMNSLRPEDTAVYYCAGTRAYGSSRLRLAETYEYWGQGTLVTVSS

SEQ ID NO: 47 - protein, 125 aa, synthetic construct
EVQLVESGGGLVQPGGSLRLSCAASGRTFASYTMGWFRQAPGKEREFVVAISKGGYKYDSVSLEARFTISRDNAKNTVYLQMNSLRPEDTAVYYCAGTRAYGSSRLRLAETYEYWGQGTLVTVSS

SEQ ID NO: 48 - protein, 125 aa, synthetic construct
EVQLVESGGGLVQPGGSLRLSCAASGRTFSSYTMGWFRQAPGKEREFVVAISKGGYKYDAVSLEARFTISRDNSKNTVYLQMNSLRAEDTAVYYCAATRAYGSSRLRLAKTYEYWGQGTLVTVSS

SEQ ID NO: 49 - protein, 125 aa, synthetic construct
EVQLVESGGGLVQPGGSLRLSCAASGRTFSSYTMGWFRQAPGKEREFVVAISKGGYKYDAVSLEARFTISRDNSKNTLYLQMNSLRPEDTAVYYCAATRAYGSSRLRLAKTYEYWGQGTLVTVSS

SEQ ID NO: 50 - protein, 125 aa, synthetic construct
EVQLVESGGGLVQPGGSLRLSCAASGRTFSSYTMGWFRQAPGKEREFVVAISKGGYKYDAVSLEARFTISRDNSKNTVYLQMNSLRPEDTAVYYCAATRAYGSSRLRLAKTYEYWGQGTLVTVSS

SEQ ID NO: 51 - protein, 125 aa, synthetic construct
EVQLVESGGGLVQPGGSLRLSCAASGRTFSSYTMGWFRQAPGKGREFVVAISKGGYKYDAVSLEARFTISRDNSKNTVYLQMNSLRPEDTAVYYCAATRAYGSSRLRLAKTYEYWGQGTLVTVSS

SEQ ID NO: 52 - protein, 125 aa, synthetic construct
EVQLVESGGGLVQPGGSLRLSCAASGRTFSSYTMGWFRQAPGKEREFVVAISKGGYKYNAVSLEARFTISRDNSKNTVYLQMNSLRPEDTAVYYCAATRAYGSSRLRLAKTYEYWGQGTLVTVSS

SEQ ID NO: 53 - protein, 125 aa, synthetic construct
EVQLVESGGGLVQPGGSLRLSCAASGRTFSSYTMGWFRQAPGKEREFVVAISKGGYKYNAVSLEARFTISRDNAKNTVYLQMNSLRPEDTAVYYCASTRAYGSSRLRLAKTYEYWGQGTLVTVSS

SEQ ID NO: 54 - protein, 125 aa, synthetic construct
EVQLVESGGGLVQPGGSLRLSCAASGRTFTSYTMGWFRQAPGKEREFVVAISKGGYKYNAVSLEARFTISRDNSKNTVYLQMNSLRPEDTAVYYCAATRAYGSSRLRLAKTYEYWGQGTLVTVSS

SEQ ID NO: 55 - protein, 125 aa, synthetic construct
EVQLVESGGGLVQPGGSLRLSCAASGRTFTSYTMGWFRQAPGKEREFVVAISKGGYKYNAVSLEARFTISRDNAKNTVYLQMNSLRPEDTAVYYCASTRAYGSSRLRLAKTYEYWGQGTLVTVSS

SEQ ID NO: 56 - protein, 125 aa, synthetic construct
EVQLVESGGGLVQPGGSLRLSCAASGRTFSSYTMGWFRQAPGKEREFVVAISKGGYKYDSVSLEARFTISRDNSKNTVYLQMNSLRAEDTAVYYCAATRAYGSSRLRLANTYEYWGQGTLVTVSS

SEQ ID NO: 57 - protein, 125 aa, synthetic construct
EVQLVESGGGLVQPGGSLRLSCAASGRTFSSYTMGWFRQAPGKEREFVVAISKGGYKYDSVSLEARFTISRDNSKNTLYLQMNSLRPEDTAVYYCAATRAYGSSRLRLANTYEYWGQGTLVTVSS

SEQ ID NO: 58 - protein, 125 aa, synthetic construct
EVQLVESGGGLVQPGGSLRLSCAASGRTFSSYTMGWFRQAPGKEREFVVAISKGGYKYDSVSLEARFTISRDNSKNTVYLQMNSLRPEDTAVYYCAATRAYGSSRLRLANTYEYWGQGTLVTVSS

SEQ ID NO: 59 - protein, 125 aa, synthetic construct
EVQLVESGGGLVQPGGSLRLSCAASGRTFTSYTMGWFRQAPGKEREFVVAISKGGYKYDSVSLEARFTISRDNSKNTVYLQMNSLRAEDTAVYYCAGTRAYGSSRLRLANTYEYWGQGTLVTVSS

SEQ ID NO: 60 - protein, 125 aa, synthetic construct
EVQLVESGGGLVQPGGSLRLSCAASGRTFTSYTMGWFRQAPGKEREFVVAISKGGYKYDSVSLEARFTISRDNSKNTLYLQMNSLRPEDTAVYYCAGTRAYGSSRLRLANTYEYWGQGTLVTVSS

SEQ ID NO: 61 - protein, 125 aa, synthetic construct
EVQLVESGGGLVQPGGSLRLSCAASGRTFTSYTMGWFRQAPGKEREFVVAISKGGYKYDSVSLEARFTISRDNAKNTVYLQMNSLRPEDTAVYYCAGTRAYGSSRLRLANTYEYWGQGTLVTVSS

SEQ ID NO: 62 - protein, 227 aa, synthetic construct
DKTHTCPPCPAPELLGGPSVFLFPPKPKDTLMISRTPEVTCVVVDVSHEDPEVKFNWYVDGVEVHNAKTKPREEQYNSTYRVVSVLTVLHQDWLNGKEYKCKVSNKALPAPIEKTISKAKGQPREPQVYTLPPSRDELTKNQVSLTCLVKGFYPSDIAVEWESNGQPENNYKTTPPVLDSDGSFFLYSKLTVDKSRWQQGNVFSCSVMHEALHNHYTQKSLSLSPGK

SEQ ID NO: 63 - protein, 227 aa, synthetic construct
DKTHTCPPCPAPELLGGPSVFLFPPKPKDTLMISRTPEVTCVVVDVSHEDPEVKFNWYVDGVEVHNAKTKPREEQYNSTYRVVSVLTVLHQDWLNGKEYKCKVSNKALPAPIEKTISKAKGQPREPQVYTLPPSREEMTKNQVSLTCLVKGFYPSDIAVEWESNGQPENNYKTTPPVLDSDGSFFLYSKLTVDKSRWQQGNVFSCSVMHEALHNHYTQKSLSLSPGK

SEQ ID NO: 64 - protein, 346 aa, synthetic construct
QLQLVESGGGSVQPGGSLRLSCEVSGRTFASYTMGWFRQAPGKEREFVVAISKGGYKYDSVSLEARFTISKDNTKNTVYLQMNSLKPEDTAVYYCAGTRAYGSSRLRLAETYEYWGQGTQVTVSSPPCPAPELLGGPSVFLFPPKPKDTLMISRTPEVTCVVVDVSHEDPEVKFNWYVDGVEVHNAKTKPREEQYNSTYRVVSVLTVLHQDWLNGKEYKCKVSNKALPAPIEKTISKAKGQPREPQVYTLPPSRDELTKNQVSLTCLVKGFYPSDIAVEWESNGQPENNYKTTPPVLDSDGSFFLYSKLTVDKSRWQQGNVFSCSVMHEALHNHYTQKSLSLSPGK

SEQ ID NO: 65 - protein, 355 aa, synthetic construct
QLQLVESGGGSVQPGGSLRLSCEVSGRTFASYTMGWFRQAPGKEREFVVAISKGGYKYDSVSLEARFTISKDNTKNTVYLQMNSLKPEDTAVYYCAGTRAYGSSRLRLAETYEYWGQGTQVTVSSGGGGSGGGSPPCPAPELLGGPSVFLFPPKPKDTLMISRTPEVTCVVVDVSHEDPEVKFNWYVDGVEVHNAKTKPREEQYNSTYRVVSVLTVLHQDWLNGKEYKCKVSNKALPAPIEKTISKAKGQPREPQVYTLPPSRDELTKNQVSLTCLVKGFYPSDIAVEWESNGQPENNYKTTPPVLDSDGSFFLYSKLTVDKSRWQQGNVFSCSVMHEALHNHYTQKSLSLSPGK

SEQ ID NO: 66 - protein, 352 aa, synthetic construct
QLQLVESGGGSVQPGGSLRLSCEVSGRTFASYTMGWFRQAPGKEREFVVAISKGGYKYDSVSLEARFTISKDNTKNTVYLQMNSLKPEDTAVYYCAGTRAYGSSRLRLAETYEYWGQGTQVTVSSDKTHTCPPCPAPELLGGPSVFLFPPKPKDTLMISRTPEVTCVVVDVSHEDPEVKFNWYVDGVEVHNAKTKPREEQYNSTYRVVSVLTVLHQDWLNGKEYKCKVSNKALPAPIEKTISKAKGQPREPQVYTLPPSRDELTKNQVSLTCLVKGFYPSDIAVEWESNGQPENNYKTTPPVLDSDGSFFLYSKLTVDKSRWQQGNVFSCSVMHEALHNHYTQKSLSLSPGK

SEQ ID NO: 67 - protein, 357 aa, synthetic construct
EVQLVESGGGLVQPGGSLRLSCAVSGRTFSSYTMGWFRQAPGKEREFVVAISKGGYKYDSVSLEARFTISRDNAKNTVYLQMNSLRPEDTAVYYCAATRAYGSSRLRLADTYEYWGQGTLVTVSSEPKSADKTHTCPPCPAPELLGGPSVFLFPPKPKDTLMISRTPEVTCVVVDVSHEDPEVKFNWYVDGVEVHNAKTKPREEQYNSTYRVVSVLTVLHQDWLNGKEYKCKVSNKALPAPIEKTISKAKGQPREPQVYTLPPSREEMTKNQVSLTCLVKGFYPSDIAVEWESNGQPENNYKTTPPVLDSDGSFFLYSKLTVDKSRWQQGNVFSCSVMHEALHNHYTQKSLSLSPGK

SEQ ID NO: 68 - protein, 23 aa, synthetic construct
MDAMKRGLCCVLLLCGAVFVSPS

SEQ ID NO: 69 - protein, 5 aa, synthetic construct
GGGGS

SEQ ID NO: 70 - protein, 4 aa, synthetic construct
SGGS

SEQ ID NO: 71 - protein, 6 aa, synthetic construct
HHHHHH

SEQ ID NO: 72 - protein, 20 aa, synthetic construct
METDTLLLWVLLLWVPGSTG

SEQ ID NO: 73 - protein, 5 aa, synthetic construct
EPKSA

SEQ ID NO: 74 - protein, 259 aa, synthetic construct
QLQLVESGGGSVQPGGSLRLSCEVSGRTFASYTMGWFRQAPGKEREFVVAISKGGYKYDSVSLEARFTISKDNTKNTVYLQMNSLKPEDTAVYYCAGTRAYGSSRLRLAETYEYWGQGTQVTVSSGGGGSGGGSQLQLVESGGGSVQPGGSLRLSCEVSGRTFASYTMGWFRQAPGKEREFVVAISKGGYKYDSVSLEARFTISKDNTKNTVYLQMNSLKPEDTAVYYCAGTRAYGSSRLRLAETYEYWGQGTQVTVSS

SEQ ID NO: 75 - protein, 221 aa, synthetic construct
PPCPAPELLGGPSVFLFPPKPKDTLMISRTPEVTCVVVDVSHEDPEVKFNWYVDGVEVHNAKTKPREEQYNSTYRVVSVLTVLHQDWLNGKEYKCKVSNKALPAPIEKTISKAKGQPREPQVYTLPPSRDELTKNQVSLTCLVKGFYPSDIAVEWESNGQPENNYKTTPPVLDSDGSFFLYSKLTVDKSRWQQGNVFSCSVMHEALHNHYTQKSLSLSPGK